European Patent Application EP 4 269 573 A1, published November 1, 2023. Title: Glycosyltransferase and method of preparing steviol glycosides using the same. Applicant: SAMYANG COPORATION. The sequence listing filed with the application follows.

SEQUENCE LISTING (16 sequences)

SEQ ID NO: 1 - protein, 461 aa, Artificial Sequence
  TaUGT amino acid sequence
MDDGSSSSSSPLRVVICPWLAFGHLLPCLDIAERLASRGHRVSFVSTPRNIARLPPVRPAVAPLVDYVALPLPRVDGLPEGAESTNDVPHDKFELLRKAFDGLAAPFSEFLHAACAEGTGKRPDWLIVDSFHHWAAAAAVENKVPCVMLLLGAANVIATWARGVSEHAAAAVGKERSAAEAPSFETERRKLMITQNASGMTVAERYFLTLMRSNLVAIRSCAEWEPESVAALTTLAGKPVVTLGLLPPSPEGGRGISKQDAAVRWLDAQRDKSVVYVALGSEVPLRVEQVHELALGLELSGASFLWALRKPPGMPDAAVLPPGFEERTRGRGLVVTGWVPQISVLAHGAVAAFLTHCGWNSTIEGLLFGQPLIMLPISSDQGPNARLMEGRKVGMQVPRNESDGSFTREDVAATVQAVAMEEDGSRVFTANAKTMQEIVADSACHERCIDGFIQQLRSYKE

SEQ ID NO: 2 - DNA, 1383 bp, Artificial Sequence
  TaUGT nucleotide sequence
atggacgacgggtcttctagctctagcagtccgctgcgtgttgttatttgcccgtggctggcttttggacacctgcttccatgcttagacattgcggaaagattagccagccgtggacacagagtatccttcgtaagtacgccgcgtaatatagcacgtttacccccggtcagaccggcagttgcgccgctggtcgattacgtagcgctacctctgcccagagtggacggacttccggaaggggctgaatctacaaacgacgtgccccatgataagttcgagcttttacgtaaggctttcgacggtttggcagcgcccttcagcgaatttctacacgcagcgtgcgcggagggcacaggcaaaagaccagattggcttattgtggattccttccaccattgggctgcggctgcggcagtggaaaataaagtcccgtgcgtcatgttacttttaggtgcagccaacgtgatcgccacttgggcacgtggcgtgtcagagcatgcggccgccgcggttggaaaagaacgtagtgccgcagaagctccatcattcgaaaccgaacgtcgtaaactgatgataactcagaatgcatcaggtatgaccgtagcagagcgttatttcctgacacttatgagatcaaacttggttgccattcgttcctgtgcagaatgggagcctgaatctgtggcggcactaaccactctggccgggaagcccgtagtgaccttaggtttgcttccaccgtctcctgagggaggaaggggtatttccaagcaagacgctgccgttaggtggctggacgctcagagggataagtccgttgtatacgtggcgttagggtctgaagttcccttgagagtggagcaggtacatgagcttgcgcttggactagagttgtcaggtgctagcttcctgtgggcgttacgtaagccacccggcatgcctgacgccgcagtcttgccgccgggttttgaagagagaaccaggggacgtggtctggttgtgactggctgggtaccacaaatcagcgtcttagcacatggcgccgttgccgcttttctgacacattgcggctggaatagtacaatcgaaggcttgctgttcggacaaccgttaatcatgctgccaatcagtagcgatcagggcccgaatgcccgtcttatggagggaagaaaagttggaatgcaggtgcctcgtaatgagtccgatggatcattcacaagagaggatgtcgctgccacagtacaagcagtagcgatggaggaggatgggagccgtgtttttacggctaatgcaaagaccatgcaagaaatagttgctgactccgcgtgtcacgaaaggtgcatcgatggatttatccaacagctaaggtcctataaagaa

SEQ ID NO: 3 - protein, 462 aa, Artificial Sequence
  EUGT11 amino acid sequence
MDSGYSSSYAAAAGMHVVICPWLAFGHLLPCLDLAQRLASRGHRVSFVSTPRNISRLPPVRPALAPLVAFVALPLPRVEGLPDGAESTNDVPHDRPDMVELHRRAFDGLAAPFSEFLGTACADWVIVDVFHHWAAAAALEHKVPCAMMLLGSAHMIASIADRRLERAETESPAAAGQGRPAAAPTFEVARMKLIRTKGSSGMSLAERFSLTLSRSSLVVGRSCVEFEPETVPLLSTLRGKPITFLGLMPPLHEGRREDGEDATVRWLDAQPAKSVVYVALGSEVPLGVEKVHELALGLELAGTRFLWALRKPTGVSDADLLPAGFEERTRGRGVVATRWVPQMSILAHAAVGAFLTHCGWNSTIEGLMFGHPLIMLPIFGDQGPNARLIEAKNAGLQVARNDGDGSFDREGVAAAIRAVAVEEESSKVFQAKAKKLQEIVADMACHERYIDGFIQQLRSYKD

SEQ ID NO: 4 - DNA, 1386 bp, Artificial Sequence
  EUGT11 nucleotide sequence
atggactccggctacagttcatcatatgctgcagccgctgggatgcacgttgtgatttgtccgtggctagcattcggtcatctgttgccgtgtttggacctggctcagaggctagcttccagaggacatcgtgtttccttcgtttctacgcctaggaatatcagtagactaccaccggtaagacctgctttagctccacttgtggcgttcgtggccctaccgttaccccgtgtagaaggattgcctgacggagcagagtctacgaatgacgtacctcacgacagacccgatatggttgaacttcacagaagagcgttcgacggtcttgctgcaccgttttccgaattccttgggacggcctgtgcggactgggtcatagtggacgtattccatcactgggctgccgcagctgccctagaacataaggttccgtgtgccatgatgttgttaggttctgctcatatgatcgcgtctattgcagaccgtaggttggagagggcagaaacggaaagtccagccgccgccggacaggggaggcccgctgcggcgccaacctttgaggtggctcgtatgaaactaattaggactaaaggttcaagcggtatgtcactggcggaaaggtttagtcttactttgtccaggtcttcattggtcgtcggtcgttcctgcgttgagtttgaacccgaaaccgttccccttctttccacgttacgtggaaaaccgattacttttcttggtcttatgccgccactgcacgagggtagaagggaagatggtgaagacgctacagttaggtggctagacgcgcaaccggctaagagcgtcgtctatgtcgcacttggctcagaggtgcccttgggggtcgagaaggtccatgagttggcgctggggttggagttggcgggtacaaggtttctttgggcccttcgtaaaccgacgggcgtatcagatgcagacctacttccggctggtttcgaggagcgtactaggggaaggggcgttgtggccacgagatgggtgccacaaatgagcatcctagctcatgccgcagtcggcgcattcttaacgcattgtggctggaattcaaccattgaagggctaatgttcggtcatccactgataatgcttcctatctttggagaccaaggtcccaatgcgcgtttgatcgaagccaagaatgctggccttcaagtcgcccgtaatgatggcgatggttcattcgacagagagggagtggcggcagcgatcagagcggttgcagtggaagaggagtccagtaaggtgtttcaggctaaggccaagaaattacaggagatagtggctgatatggcttgccacgagagatatatcgacggctttatacaacagctacgttcttataaggac

SEQ ID NO: 5 - protein, 463 aa, Artificial Sequence
  HvUGT amino acid sequence
MDGDGNSSSSSSPLHVVICPWLALGHLLPCLDIAERLASRGHRVSFVSTPRNIARLPPLRPAVAPLVEFVALPLPHVDGLPEGAESTNDVPYDKFELHRKAFDGLAAPFSEFLRAACAEGAGSRPDWLIVDTFHHWAAAAAVENKVPCVMLLLGAATVIAGFARGVSEHAAAAVGKERPAAEAPSFETERRKLMTTQNASGMTVAERYFLTLMRSDLVAIRSCAEWEPESVAALTTLAGKPVVPLGLLPPSPEGGRGVSKEDAAVRWLDAQPAKSVVYVALGSEVPLRAEQVHELALGLELSGARFLWALRKPTDAPDAAVLPPGFEERTRGRGLVVTGWVPQIGVLAHGAVAAFLTHCGWNSTIEGLLFGHPLIMLPISSDQGPNARLMEGRKVGMQVPRDESDGSFRREDVAATVRAVAVEEDGRRVFTANAKKMQEIVADGACHERCIDGFIQQLRSYKA

SEQ ID NO: 6 - DNA, 1389 bp, Artificial Sequence
  HvUGT nucleotide sequence
atggacggcgacggaaacagttcatcaagttctagtcctctgcatgttgttatatgtccctggctagctcttgggcatcttcttccttgtttggacattgcggaaagactggcctcaagaggacacagggtcagcttcgtatccacgccaagaaatattgcccgtctacccccgcttaggccagcggtggctcccttagtagagttcgttgctctacctctgcctcacgtggacgggttacctgaaggggctgaaagtacaaacgatgtaccctatgacaagtttgaacttcaccgtaaggcgttcgacgggctggccgctccttttagcgagttcttgagagctgcttgtgccgagggggctggttcccgtcctgattggctaatcgtggatacattccatcactgggcagcggcagccgccgttgaaaataaagtgccatgcgtgatgttactgcttggtgcagccaccgttattgccgggttcgcaagaggggtcagtgagcacgccgccgctgcagtcggtaaagagagaccggccgctgaagccccgagttttgagacggagagacgtaaacttatgaccactcagaatgcaagtggtatgacggttgcagaaaggtatttcctaaccttaatgcgtagtgacttggtcgcaatacgtagctgcgccgagtgggagcccgagtctgtcgcggcgttgacaaccttagcaggcaagcccgtcgttcctttaggcttgctgccaccgtctccagagggggggagaggcgtttccaaggaggacgccgcggttcgttggttggatgcgcaacccgcgaagagcgtcgtgtatgtcgcgttaggcagtgaggttccattgagagctgaacaagtccacgagttggcgcttggtttagaattatctggcgctaggtttttatgggcgctaaggaaacccaccgacgcgccagatgccgcggtattgccgccagggtttgaggaaaggactcgtggcagagggcttgtcgtgaccggttgggtgcctcaaatcggcgttcttgctcatggtgccgtagcagcattcttgactcattgtggctggaattcaaccatcgaggggctgctgtttggtcacccgttgatcatgctgccaataagctccgaccaaggacccaatgctcgtttgatggaaggcagaaaagtggggatgcaggtgcccagagacgaaagcgatgggagttttaggagagaagatgtggcagctactgttcgtgctgtagcggtggaggaagatggcagaagggtttttacagctaatgcgaagaagatgcaagaaatagtagccgacggggcttgtcacgagagatgcatcgatggatttatccaacaactgcgttcctacaaagct

SEQ ID NO: 7 - DNA, 31 bp, Artificial Sequence
  Forward primer for CYC1 terminator
tgattgtcgatatcatgtaattagttatgtc

SEQ ID NO: 8 - DNA, 28 bp, Artificial Sequence
  Reverse primer for GAL10 promoter
catcaattcttactttttttttggatgg

SEQ ID NO: 9 - DNA, 44 bp, Artificial Sequence
  Forward primer for connecting TaUGT and GAL10 promoter
catccaaaaaaaaagtaagaattgatggacgacgggtcttctag

SEQ ID NO: 10 - DNA, 48 bp, Artificial Sequence
  Reverse primer for connecting TaUGT and CYC1 terminator
ctaattacatgatatcgacaatcattctttataggaccttagctgttg

SEQ ID NO: 11 - DNA, 44 bp, Artificial Sequence
  Forward primer for connecting EUGT11 and GAL10 promoter
catccaaaaaaaaagtaagaattgatggactccggctacagttc

SEQ ID NO: 12 - DNA, 45 bp, Artificial Sequence
  Reverse primer for connecting EUGT11 and CYC1 terminator
ctaattacatgatatcgacaattagtccttataagaacgtagctg

SEQ ID NO: 13 - DNA, 42 bp, Artificial Sequence
  Forward primer for connecting HvUGT and GAL10 promoter
catccaaaaaaaaagtaagaattgatggacggcgacggaaac

SEQ ID NO: 14 - DNA, 45 bp, Artificial Sequence
  Reverse primer for connecting HvUGT and CYC1 terminator
ctaattacatgatatcgacaatcaagctttgtaggaacgcagttg

SEQ ID NO: 15 - DNA, 18 bp, Artificial Sequence
  Forward primer for GAL10 promoter
ggatccatcgcttcgctg

SEQ ID NO: 16 - DNA, 20 bp, Artificial Sequence
  Reverse primer for CYC1 terminator
gcaaattaaagccttcgagc